European Patent Application EP 4 410 810 A1, published August 7, 2024. Title: Peptide having hair loss preventing activity or hair growth promoting activity and use thereof. Applicant: CAREGENE CO., LTD. Application KR. The sequence listing filed with the application follows.

SEQUENCE LISTING (17 sequences)

SEQ ID NO: 1 - protein, 9 aa, synthetic construct
GCGLFVAAC

SEQ ID NO: 2 - DNA, 20 bp, synthetic construct
  source 1..20: mol_type = other DNA
ccagctattgtaacacctca

SEQ ID NO: 3 - DNA, 20 bp, synthetic construct
  source 1..20: mol_type = other DNA
ttcagatgtaggcagctgtc

SEQ ID NO: 4 - DNA, 28 bp, synthetic construct
  source 1..28: mol_type = other DNA
accttcgttgccctctgtgccacagatg

SEQ ID NO: 5 - DNA, 21 bp, synthetic construct
  source 1..21: mol_type = other DNA
aggcccggaggcagtccgggt

SEQ ID NO: 6 - DNA, 20 bp, synthetic construct
  source 1..20: mol_type = other DNA
ggagccaaaagggtcatcat

SEQ ID NO: 7 - DNA, 20 bp, synthetic construct
  source 1..20: mol_type = other DNA
gtgatggcatggactgtggt

SEQ ID NO: 8 - DNA, 20 bp, synthetic construct
  source 1..20: mol_type = other DNA
gatcatcgagctgagacgca

SEQ ID NO: 9 - DNA, 20 bp, synthetic construct
  source 1..20: mol_type = other DNA
ctggccccagggtatctagt

SEQ ID NO: 10 - DNA, 20 bp, synthetic construct
  source 1..20: mol_type = other DNA
ccctcaaggatgccaggaac

SEQ ID NO: 11 - DNA, 19 bp, synthetic construct
  source 1..19: mol_type = other DNA
cactgctacctccggcaag

SEQ ID NO: 12 - DNA, 20 bp, synthetic construct
  source 1..20: mol_type = other DNA
ccaaatccgcaccaaggtca

SEQ ID NO: 13 - DNA, 21 bp, synthetic construct
  source 1..21: mol_type = other DNA
gtattgattgccaggaggggg

SEQ ID NO: 14 - DNA, 20 bp, synthetic construct
  source 1..20: mol_type = other DNA
cgcggcgtatccgtgtcctc

SEQ ID NO: 15 - DNA, 24 bp, synthetic construct
  source 1..24: mol_type = other DNA
agcctgttccgtctcaaacttggt

SEQ ID NO: 16 - DNA, 20 bp, synthetic construct
  source 1..20: mol_type = other DNA
cggtcaagtcggaaaattca

SEQ ID NO: 17 - DNA, 20 bp, synthetic construct
  source 1..20: mol_type = other DNA
gaggagctgggatgtggtaa